European Patent Application EP 4 495 138 A1, published January 22, 2025. Title: ANTIBODIES BINDING B7-H3 AND USES THEREOF. Applicant: Beijing Mabworks Biotech Co., Ltd Biocytogen Pharmaceuticals (Beijing) Co., Ltd. Application EP22931427.3. The sequence listing filed with the application follows.

SEQUENCE LISTING (75 sequences)

SEQ ID NO: 1 - protein, 7 aa, Artificial sequence
  6B5 and 15F11's VH-CDR1
SGGYYWS

SEQ ID NO: 2 - protein, 16 aa, Artificial sequence
  6B5's VH-CDR2
YIYYSGGTYYSPSLKS

SEQ ID NO: 3 - protein, 10 aa, Artificial sequence
  6B5's VH-CDR3
RAGYSSSFDS

SEQ ID NO: 4 - protein, 16 aa, Artificial sequence
  6B5's VL-CDR1
RSSQSLLYSNGYTYLD

SEQ ID NO: 5 - protein, 7 aa, Artificial sequence
  6B5's VL-CDR2
LGFNRAS

SEQ ID NO: 6 - protein, 9 aa, Artificial sequence
  6B5's VL-CDR3
MQGLQTPYT

SEQ ID NO: 7 - protein, 16 aa, Artificial sequence
  15F11's VH-CDR2
YIYYSGSTYYNPSLKS

SEQ ID NO: 8 - protein, 11 aa, Artificial sequence
  15F11's VH-CDR3
ERIAVAGYFDY

SEQ ID NO: 9 - protein, 12 aa, Artificial sequence
  15F11 and 10F7's VL-CDR1
RASQSVSSSYLA

SEQ ID NO: 10 - protein, 7 aa, Artificial sequence
  15F11's VL-CDR2
GASTRAT

SEQ ID NO: 11 - protein, 9 aa, Artificial sequence
  15F11's VL-CDR3
QQYGSSPLT

SEQ ID NO: 12 - protein, 7 aa, Artificial sequence
  10D7's VH-CDR1
RSSYYWG

SEQ ID NO: 13 - protein, 16 aa, Artificial sequence
  10D7's VH-CDR2
NIFYAGSTYYNPSLKS

SEQ ID NO: 14 - protein, 11 aa, Artificial sequence
  10D7's VH-CDR3
RITGTTGWFDP

SEQ ID NO: 15 - protein, 11 aa, Artificial sequence
  10D7's VL-CDR1
RASQGIRNDLG

SEQ ID NO: 16 - protein, 7 aa, Artificial sequence
  10D7's VL-CDR2
AASTLQS

SEQ ID NO: 17 - protein, 9 aa, Artificial sequence
  10D7's VL-CDR3
LQDYNYPRT

SEQ ID NO: 18 - protein, 7 aa, Artificial sequence
  10F7's VH-CDR1
SSSAAWN

SEQ ID NO: 19 - protein, 18 aa, Artificial sequence
  10F7's VH-CDR2
RTYYRSKWYNDFAVSVKS

SEQ ID NO: 20 - protein, 15 aa, Artificial sequence
  10F7's VH-CDR3
DLITLVRGVILPFDY

SEQ ID NO: 21 - protein, 7 aa, Artificial sequence
  10F7's VL-CDR2
GASSRAT

SEQ ID NO: 22 - protein, 8 aa, Artificial sequence
  10F7's VL-CDR3
QQYGSSHT

SEQ ID NO: 23 - protein, 5 aa, Artificial sequence
  10F5's VH-CDR1
SQAIS

SEQ ID NO: 24 - protein, 17 aa, Artificial sequence
  10F5's VH-CDR2
RIIPMLGIGDYAQSFQG

SEQ ID NO: 25 - protein, 16 aa, Artificial sequence
  10F5's VH-CDR3
EGIAALGTNYYYGMDV

SEQ ID NO: 26 - protein, 11 aa, Artificial sequence
  10F5's VL-CDR1
RASQGISRWLA

SEQ ID NO: 27 - protein, 7 aa, Artificial sequence
  10F5's VL-CDR2
VASSLQS

SEQ ID NO: 28 - protein, 9 aa, Artificial sequence
  10F5's VL-CDR3
QQANSFPFT

SEQ ID NO: 29 - protein, 120 aa, Artificial sequence
  6B5's VH
QVQLVESGPGLVKPSQTLSLTCTVSDGSISSGGYYWSWIRQHPGKGLEWIGYIYYSGGTYYSPSLKSRVTISVDTSKNQFSLKLTSVTAADTAVYYCARRAGYSSSFDSWGQGILVTVSS

SEQ ID NO: 30 - protein, 112 aa, Artificial sequence
  6B5's VL
EIVLTQSPLSLPVTPGEPASISCRSSQSLLYSNGYTYLDWYLQKPGQSPQFLIYLGFNRASGVPDRFSGSGSGTDFTLKISRVEAEDVGVYYCMQGLQTPYTFGQGTKLEIK

SEQ ID NO: 31 - protein, 121 aa, Artificial sequence
  15F11's VH
EVQLVQSGPGLVKPSQTLSLTCTVSGGSINSGGYYWSWIRQHPGKGLEWIGYIYYSGSTYYNPSLKSRVTISIDTSKNQFSLKLSSVTAADTAVYYCARERIAVAGYFDYWGQGTLVTVSS

SEQ ID NO: 32 - protein, 108 aa, Artificial sequence
  15F11's VL
EIVMTQSPGTLSLSPGESATLSCRASQSVSSSYLAWYQQKPGQAPRLLIYGASTRATGIPDRFSGSGSGTDFTLTISRLEPEDFAVYFCQQYGSSPLTFGGETKVEIK

SEQ ID NO: 33 - protein, 121 aa, Artificial sequence
  10D7's VH
QVQLVQSGPGLVKPSETLSLTCTVSGGSISRSSYYWGWIRQPPGKGLEWIGNIFYAGSTYYNPSLKSRVTISVDTSKNQFSLKLSSVTAADTAVYYCARRITGTTGWFDPWGQGTLVTVSS

SEQ ID NO: 34 - protein, 107 aa, Artificial sequence
  10D7's VL
DIQLTQSPSSLSASVGDRVTITCRASQGIRNDLGWYQQKPGKAPKLLIYAASTLQSGVPSRFSGSGSGTDFTLTISSLQPEDFATYYCLQDYNYPRTFGQGTKVEIK

SEQ ID NO: 35 - protein, 127 aa, Artificial sequence
  10F7's VH
QVQLVQSGPGLVKPSQTLSLTCAISGDSVSSSSAAWNWIRQSPSRGLEWLGRTYYRSKWYNDFAVSVKSRITINPDTSKNQFSLQLNSVTPEDTAVYYCARDLITLVRGVILPFDYWGQGTLVTVSS

SEQ ID NO: 36 - protein, 107 aa, Artificial sequence
  10F7's VL
EIVLTQSPGTLSLSPGERATLSCRASQSVSSSYLAWYQQRPGQAPRLLIYGASSRATGIPDRFSGSGSGTDFTLTISRLEPEDFAVYYCQQYGSSHTFGQGTNLEIK

SEQ ID NO: 37 - protein, 125 aa, Artificial sequence
  10F5's VH
QVQLVQSGAEVKKPGSSVKVSCKASGGTFSSQAISWVRQAPGQGLEWMGRIIPMLGIGDYAQSFQGRVTITADKSTSTAYLEVSSLGSEDTAVYYCAREGIAALGTNYYYGMDVWGQGTAVTVSS

SEQ ID NO: 38 - protein, 107 aa, Artificial sequence
  10F5's VL
EIVMTQSPSSVSASVGDRVTITCRASQGISRWLAWYQQKPGKAPKLLIYVASSLQSGVPSRFSGSGSGTDFTLTISSLQPEDFATYYCQQANSFPFTFGPGTKVDIR

SEQ ID NO: 39 - protein, 122 aa, Artificial sequence
  Enoblituzumab's VH
EVQLVESGGGLVQPGGSLRLSCAASGFTFSSFGMHWVRQAPGKGLEWVAYISSDSSAIYYADTVKGRFTISRDNAKNSLYLQMNSLRDEDTAVYYCGRGRENIYYGSRLDYWGQGTTVTVSS

SEQ ID NO: 40 - protein, 107 aa, Artificial sequence
  Enoblituzumab's VL
DIQLTQSPSFLSASVGDRVTITCKASQNVDTNVAWYQQKPGKAPKALIYSASYRYSGVPSRFSGSGSGTDFTLTISSLQPEDFATYYCQQYNNYPFTFGQGTKLEIK

SEQ ID NO: 41 - protein, 118 aa, Artificial sequence
  Omburtamab's VH
QVQLQQSGAELVKPGASVKLSCKASGYTFTNYDINWVRQRPEQGLEWIGWIFPGDGSTQYNEKFKGKATLTTDTSSSTAYMQLSRLTSEDSAVYFCARQTTATWFAYWGQGTLVTVSA

SEQ ID NO: 42 - protein, 107 aa, Artificial sequence
  Omburtamab's VL
DIVMTQSPATLSVTPGDRVSLSCRASQSISDYLHWYQQKSHESPRLLIKYASQSISGIPSRFSGSGSGSDFTLSINSVEPEDVGVYYCQNGHSFPLTFGAGTKLELK

SEQ ID NO: 43 - protein, 330 aa, Artificial sequence
  human IgG1 constant region (wildtype)
ASTKGPSVFPLAPSSKSTSGGTAALGCLVKDYFPEPVTVSWNSGALTSGVHTFPAVLQSSGLYSLSSVVTVPSSSLGTQTYICNVNHKPSNTKVDKKVEPKSCDKTHTCPPCPAPELLGGPSVFLFPPKPKDTLMISRTPEVTCVVVDVSHEDPEVKFNWYVDGVEVHNAKTKPREEQYNSTYRVVSVLTVLHQDWLNGKEYKCKVSNKALPAPIEKTISKAKGQPREPQVYTLPPSREEMTKNQVSLTCLVKGFYPSDIAVEWESNGQPENNYKTTPPVLDSDGSFFLYSKLTVDKSRWQQGNVFSCSVMHEALHNHYTQKSLSLSPGK

SEQ ID NO: 44 - protein, 330 aa, Artificial sequence
  human IgG1-Mut constant region
ASTKGPSVFPLAPSSKSTSGGTAALGCLVKDYFPEPVTVSWNSGALTSGVHTFPAVLQSSGLYSLSSVVTVPSSSLGTQTYICNVNHKPSNTKVDKRVEPKSCDKTHTCPPCPAPELVGGPSVFLLPPKPKDTLMISRTPEVTCVVVDVSHEDPEVKFNWYVDGVEVHNAKTKPPEEQYNSTLRVVSVLTVLHQDWLNGKEYKCKVSNKALPAPIEKTISKAKGQPREPQVYTLPPSREEMTKNQVSLTCLVKGFYPSDIAVEWESNGQPENNYKTTPLVLDSDGSFFLYSKLTVDKSRWQQGNVFSCSVMHEALHNHYTQKSLSLSPGK

SEQ ID NO: 45 - protein, 107 aa, Artificial sequence [sequence omitted]

SEQ ID NO: 46 - protein, 9 aa, Artificial sequence
  6B5's VH-CDR1
DGSISSGGY

SEQ ID NO: 47 - protein, 5 aa, Artificial sequence
  6B5's VH-CDR2
YYSGG

SEQ ID NO: 48 - protein, 10 aa, Artificial sequence
  6B5's VH-CDR3
RAGYSSSFDS

SEQ ID NO: 49 - protein, 16 aa, Artificial sequence
  6B5's VL-CDR1
RSSQSLLYSNGYTYLD

SEQ ID NO: 50 - protein, 7 aa, Artificial sequence
  6B5's VL-CDR2
LGFNRAS

SEQ ID NO: 51 - protein, 9 aa, Artificial sequence
  6B5's VL-CDR3
MQGLQTPYT

SEQ ID NO: 52 - protein, 9 aa, Artificial sequence
  15F11's VH-CDR1
GGSINSGGY

SEQ ID NO: 53 - protein, 5 aa, Artificial sequence
  15F11's VH-CDR2
YYSGS

SEQ ID NO: 54 - protein, 11 aa, Artificial sequence
  15F11's VH-CDR3
ERIAVAGYFDY

SEQ ID NO: 55 - protein, 12 aa, Artificial sequence
  15F11's VL-CDR1
RASQSVSSSYLA

SEQ ID NO: 56 - protein, 7 aa, Artificial sequence
  15F11's VL-CDR2
GASTRAT

SEQ ID NO: 57 - protein, 9 aa, Artificial sequence
  15F11's VL-CDR3
QQYGSSPLT

SEQ ID NO: 58 - protein, 9 aa, Artificial sequence
  10D7's VH-CDR1
GGSISRSSY

SEQ ID NO: 59 - protein, 5 aa, Artificial sequence
  10D7's VH-CDR2
FYAGS

SEQ ID NO: 60 - protein, 11 aa, Artificial sequence
  10D7's VH-CDR3
RITGTTGWFDP

SEQ ID NO: 61 - protein, 11 aa, Artificial sequence
  10D7's VL-CDR1
RASQGIRNDLG

SEQ ID NO: 62 - protein, 7 aa, Artificial sequence
  10D7's VL-CDR2
AASTLQS

SEQ ID NO: 63 - protein, 9 aa, Artificial sequence
  10D7's VL-CDR3
LQDYNYPRT

SEQ ID NO: 64 - protein, 9 aa, Artificial sequence
  10F7's VH-CDR1
GDSVSSSSA

SEQ ID NO: 65 - protein, 7 aa, Artificial sequence
  10F7's VH-CDR2
YYRSKWY

SEQ ID NO: 66 - protein, 15 aa, Artificial sequence
  10F7's VH-CDR3
DLITLVRGVILPFDY

SEQ ID NO: 67 - protein, 12 aa, Artificial sequence
  10F7's VL-CDR1
RASQSVSSSYLA

SEQ ID NO: 68 - protein, 7 aa, Artificial sequence
  10F7's VL-CDR2
GASSRAT

SEQ ID NO: 69 - protein, 8 aa, Artificial sequence
  10F7's VL-CDR3
QQYGSSHT

SEQ ID NO: 70 - protein, 7 aa, Artificial sequence
  10F5's VH-CDR1
GGTFSSQ

SEQ ID NO: 71 - protein, 6 aa, Artificial sequence
  10F5's VH-CDR2
IPMLGI

SEQ ID NO: 72 - protein, 16 aa, Artificial sequence
  10F5's VH-CDR3
EGIAALGTNYYYGMDV

SEQ ID NO: 73 - protein, 11 aa, Artificial sequence
  10F5's VL-CDR1
RASQGISRWLA

SEQ ID NO: 74 - protein, 7 aa, Artificial sequence
  10F5's VL-CDR2
VASSLQS

SEQ ID NO: 75 - protein, 9 aa, Artificial sequence
  10F5's VL-CDR3
QQANSFPFT